European Patent Application EP 4 450 522 A2, published October 23, 2024. Title: Antibody against Ox40 and medical use thereof. Applicant: Innolake Biopharma (Hangzhou)Co., Ltd. Application CN PCT/CN2023/074425, filed February 3, 2022. The sequence listing filed with the application follows.

SEQUENCE LISTING (54 sequences)

SEQ ID NO: 1 - protein, 119 aa, synthetic construct
  REGION 1..119: note = 1G2 Heavy chain variable region
EVQLQQSGPDLVKPGASVKMSCKASGYRFTSYVMHWVKQRPGQGLEWIGYINPYNDNTRYNEKFKGKATLTSDKSSSTAYMELSSLTSEDSAVYYCAAYYGDYVYLDYWGQGTTLTVSS

SEQ ID NO: 2 - protein, 109 aa, synthetic construct
  REGION 1..109: note = 1G2 Light chain variable region
DIQMTQTTSSLSASLGDRVTISCRASQDINNYLNWYQQKPDGTVKLLIYYTSRLHSGVPSRFSGSGSGTDYSLIISNLEQEDIATYFCQQGNTLPWTFGGGTKLEIKRA

SEQ ID NO: 3 - protein, 120 aa, synthetic construct
  REGION 1..120: note = 3G4 Heavy chain variable region
EVQLQQSGPELVKPGTSVKMSCKASGYRFTSYVLHWVRRKPGQGLEWIGYVNPFNDNTRYNEKFKAKATLTSDKSSSTAYMDLVSLTSEDSAVYYCSRGLYDYSYVMDYWGQGTSVTVSS

SEQ ID NO: 4 - protein, 109 aa, synthetic construct
  REGION 1..109: note = 3G4 Light chain variable region
DIQMTQTTSSLSASLGDGVTITCQASQDIRNYLNWYQQKPDGTIKLLIYHTSKLHSGVPSRFSGGGSGTDFSLTISNLDQEDIATYFCQQSQTLPYTFGGGTKLEIKRA

SEQ ID NO: 5 - protein, 119 aa, synthetic construct
  REGION 1..119: note = 9G7 Heavy chain variable region
EVKLVESGGGLVQPGGSLKLSCAASGFTFSDYYMYWVRQTPEKRLEWVAYISNGDISTYYPDTVKGRFTISRDNAKNTLYLQMSRLKSEDTAMYYCARDDGYSAWFAYWGQGTLVTVSA

SEQ ID NO: 6 - protein, 115 aa, synthetic construct
  REGION 1..115: note = 9G7 Light chain variable region
DIVMTQSPSSLAMSVGQKVTLSCKSSQSLLNSSNQKNYLAWYQQRPGQSPKLLVYFASTRESGVPDRFIGSGSGTDFTLTISSVQAEDLADYFCQQHYYTPFTFGSGTKLEIKRA

SEQ ID NO: 7 - protein, 119 aa, synthetic construct
  REGION 1..119: note = 177G5 Heavy chain variable region
EVQLVESGGGLVKPGGSLKLSCAASGFTFSDFYMYWVRQTPEKRLEWVATISDGGSYTYYPDIVKGRFTISRDNAKNNLNLQMSSLKSDDTAMYYCTTKNGNHIGFAYWGQGTLVTVSA

SEQ ID NO: 8 - protein, 109 aa, synthetic construct
  REGION 1..109: note = 177G5 Light chain variable region
DIQMTQSPASLSVSVGETVTITCRASENIYSNLAWYQQKQGKSPQLLVYAATNLADGVPSRFSGSGSGTQYSLKINSLQSEDFGSYYCQHFWGIPWTFGGGTKLEIKRA

SEQ ID NO: 9 - protein, 115 aa, synthetic construct
  REGION 1..115: note = 118A10 Heavy chain variable region
EVKLDETGGGLVQPGRPMKLSCVASGFTFSDYWLNWVRQSPEKGLEWVAQIRNKPYHYETFYSESVKGRFTISRDDSKSSVYLQMNDLRGEDTGIYYCTGYFDYWGQGTTLTVSS

SEQ ID NO: 10 - protein, 113 aa, synthetic construct
  REGION 1..113: note = 118A10 Light chain variable region
DIVLTQSPASLTISLGQRATISCRASQSVSTSTYSYIHWYQQKPGQPPRLLIKYASNLESGVPARFSGSGSGTDFTLNIHPVEEEDTATYYCQHSWGIPPTFGGGTKLEIKRA

SEQ ID NO: 11 - protein, 115 aa, synthetic construct
  REGION 1..115: note = 119H2 Heavy chain variable region
EVKLDATGGGLVQPGRPMKLSCVASGFTFSDYWMNWVRQSPEKGLEWVAQIRNKPYNYETFYSDSVKGRFTISRDDSKSSVYLQMNNLRAEDMGIYYCTGYFDYWGQGTTLTVSS

SEQ ID NO: 12 - protein, 113 aa, synthetic construct
  REGION 1..113: note = 119H2 Light chain variable region
DIVLTQSPASLAVSLGQRATISCRASQSVSTSSYSYMHWYQQKPGQPPKLLIKYASNLESGVPARFSGSGSGTDFTLNIHPVEEEDTATYYCQHSWGIPPTFGGGTKLEIKRA

SEQ ID NO: 13 - protein, 5 aa, synthetic construct
  REGION 1..5: note = 1G2 Heavy chain CDR1
SYVMH

SEQ ID NO: 14 - protein, 17 aa, synthetic construct
  REGION 1..17: note = 1G2 Heavy chain CDR2
YINPYNDNTRYNEKFKG

SEQ ID NO: 15 - protein, 10 aa, synthetic construct
  REGION 1..10: note = 1G2 Heavy chain CDR3
YYGDYVYLDY

SEQ ID NO: 16 - protein, 11 aa, synthetic construct
  REGION 1..11: note = 1G2 Light chain CDR1
RASQDINNYLN

SEQ ID NO: 17 - protein, 7 aa, synthetic construct
  REGION 1..7: note = 1G2 Light chain CDR2
YTSRLHS

SEQ ID NO: 18 - protein, 9 aa, synthetic construct
  REGION 1..9: note = 1G2 Light chain CDR3
QQGNTLPWT

SEQ ID NO: 19 - protein, 5 aa, synthetic construct
  REGION 1..5: note = 3G4 Heavy chain CDR1
SYVLH

SEQ ID NO: 20 - protein, 17 aa, synthetic construct
  REGION 1..17: note = 3G4 Heavy chain CDR2
YVNPFNDNTRYNEKFKA

SEQ ID NO: 21 - protein, 11 aa, synthetic construct
  REGION 1..11: note = 3G4 Heavy chain CDR3
GLYDYSYVMDY

SEQ ID NO: 22 - protein, 11 aa, synthetic construct
  REGION 1..11: note = 3G4 Light chain CDR1
QASQDIRNYLN

SEQ ID NO: 23 - protein, 7 aa, synthetic construct
  REGION 1..7: note = 3G4 Light chain CDR2
HTSKLHS

SEQ ID NO: 24 - protein, 9 aa, synthetic construct
  REGION 1..9: note = 3G4 Light chain CDR3
QQSQTLPYT

SEQ ID NO: 25 - protein, 5 aa, synthetic construct
  REGION 1..5: note = 9G7 Heavy chain CDR1
DYYMY

SEQ ID NO: 26 - protein, 17 aa, synthetic construct
  REGION 1..17: note = 9G7 Heavy chain CDR2
YISNGDISTYYPDTVKG

SEQ ID NO: 27 - protein, 10 aa, synthetic construct
  REGION 1..10: note = 9G7 Heavy chain CDR3
DDGYSAWFAY

SEQ ID NO: 28 - protein, 17 aa, synthetic construct
  REGION 1..17: note = 9G7 Light chain CDR1
KSSQSLLNSSNQKNYLA

SEQ ID NO: 29 - protein, 7 aa, synthetic construct
  REGION 1..7: note = 9G7 Light chain CDR2
FASTRES

SEQ ID NO: 30 - protein, 9 aa, synthetic construct
  REGION 1..9: note = 9G7 Light chain CDR3
QQHYYTPFT

SEQ ID NO: 31 - protein, 5 aa, synthetic construct
  REGION 1..5: note = 177G5 Heavy chain CDR1
DFYMY

SEQ ID NO: 32 - protein, 17 aa, synthetic construct
  REGION 1..17: note = 177G5 Heavy chain CDR2
TISDGGSYTYYPDIVKG

SEQ ID NO: 33 - protein, 10 aa, synthetic construct
  REGION 1..10: note = 177G5 Heavy chain CDR3
KNGNHIGFAY

SEQ ID NO: 34 - protein, 11 aa, synthetic construct
  REGION 1..11: note = 177G5 Light chain CDR1
RASENIYSNLA

SEQ ID NO: 35 - protein, 7 aa, synthetic construct
  REGION 1..7: note = 177G5 Light chain CDR2
AATNLAD

SEQ ID NO: 36 - protein, 9 aa, synthetic construct
  REGION 1..9: note = 177G5 Light chain CDR3
QHFWGIPWT

SEQ ID NO: 37 - protein, 5 aa, synthetic construct
  REGION 1..5: note = 118A10 Heavy chain CDR1
DYWLN

SEQ ID NO: 38 - protein, 19 aa, synthetic construct
  REGION 1..19: note = 118A10 Heavy chain CDR2
QIRNKPYHYETFYSESVKG

SEQ ID NO: 39 - protein, 4 aa, synthetic construct
  REGION 1..4: note = 118A10 Heavy chain CDR3
YFDY

SEQ ID NO: 40 - protein, 15 aa, synthetic construct
  REGION 1..15: note = 118A10 Light chain CDR1
RASQSVSTSTYSYIH

SEQ ID NO: 41 - protein, 7 aa, synthetic construct
  REGION 1..7: note = 118A10 Light chain CDR2
YASNLES

SEQ ID NO: 42 - protein, 9 aa, synthetic construct
  REGION 1..9: note = 118A10 Light chain CDR3
QHSWGIPPT

SEQ ID NO: 43 - protein, 5 aa, synthetic construct
  REGION 1..5: note = 119H2 Heavy chain CDR1
DYWMN

SEQ ID NO: 44 - protein, 19 aa, synthetic construct
  REGION 1..19: note = 119H2 Heavy chain CDR2
QIRNKPYNYETFYSDSVKG

SEQ ID NO: 45 - protein, 4 aa, synthetic construct
  REGION 1..4: note = 119H2 Heavy chain CDR3
YFDY

SEQ ID NO: 46 - protein, 15 aa, synthetic construct
  REGION 1..15: note = 119H2 Light chain CDR1
RASQSVSTSSYSYMH

SEQ ID NO: 47 - protein, 7 aa, synthetic construct
  REGION 1..7: note = 119H2 Light chain CDR2
YASNLES

SEQ ID NO: 48 - protein, 9 aa, synthetic construct
  REGION 1..9: note = 119H2 Light chain CDR3
QHSWGIPPT

SEQ ID NO: 49 - protein, 120 aa, synthetic construct
  REGION 1..120: note = hu3G4 humanized heavy chain
QVQLVQSGAEVKKPGASVKVSCKASGYRFTSYVLHWVRQAPGQRLEWIGYVNPFNDNTRYNEKFKARATLTSDKSASTAYMELSSLRSEDTAVYYCSRGLYDYSYVMDYWGQGTLVTVSS

SEQ ID NO: 50 - protein, 107 aa, synthetic construct
  REGION 1..107: note = hu3G4 humanized light chain
DIQMTQSPSSLSASVGDRVTITCQASQDIRNYLNWYQQKPGKAPKLLIYHTSKLHSGVPSRFSGSGSGTDFTFTISSLQPEDIATYYCQQSNTLPYTFGQGTKLEIK

SEQ ID NO: 51 - protein, 119 aa, synthetic construct
  REGION 1..119: note = hu9G7 humanized heavy chain
EVQLVESGGGLVQPGGSLRLSCAASGFTFSDYYMYWVRQAPGKGLEWVAYISNGDISTYYPDTVKGRFTISRDNAKNSLYLQMNSLRAEDTAVYYCARDDGYSAWFAYWGQGTTVTVSS

SEQ ID NO: 52 - protein, 113 aa, synthetic construct
  REGION 1..113: note = hu9G7 humanized light chain
DIVMTQSPDSLAVSLGERATINCKSSQSLLNSSNQKNYLAWYQQKPGQPPKLLVYFASTRESGVPDRFSGSGSGTDFTLTISSLQAEDVAVYYCQQHYYTPFTFGQGTKLEIK

SEQ ID NO: 53 - protein, 119 aa, synthetic construct
  REGION 1..119: note = hu177G5 humanized heavy chain
QVQLVESGGGLVKPGGSLRLSCAASGFTFSDFYMYWIRQAPGKGLEWVATISDGGSYTYYPDIVKGRFTISRDNAKNSLNLQMNSLRAEDTAVYYCTTKNGNHIGFAYWGQGTTVTVSS

SEQ ID NO: 54 - protein, 107 aa, synthetic construct
  REGION 1..107: note = hu177G5 humanized light chain
DIQMTQSPSSLSASVGDRVTITCRASENIYSNLAWYQQKPGKAPKLLVYAATNLADGVPSRFSGSGSGTDYTLTISSLQPEDFATYYCQHFWGIPWTFGGGTKVEIK